European Patent Specification EP 4 015 633 B1, published April 22, 2026. Title: Precise Deletion of Chromosomal Sequences In Vivo and Treatment of Nucleotide Repeat Expansion Disorders Using Engineered Nucleases. Applicant: Precision Biosciences, Inc. The sequence listing filed with the application follows.

SEQUENCE LISTING (250 sequences)

SEQ ID NO: 1 - protein, 163 aa, Chlamydomonas reinhardtii
MNTKYNKEFLLYLAGFVDGDGSIIAQIKPNQSYKFKHQLSLAFQVTQKTQRRWFLDKLVDEIGVGYVRDRGSVSDYILSEIKPLHNFLTQLQPFLKLKQKQANLVLKIIWRLPSAKESPDKFLEVCTWVDQIAALNDSKTRKTTSETVRAVLDSLSEKKKSSP

SEQ ID NO: 2 - DNA, 22 bp, Homo sapiens
gggccgacggcgagcgcgggcg

SEQ ID NO: 3 - DNA, 109 bp, Homo sapiens
acttccggtggagggccgcctctgagcgggcggcgggccgacggcgagcgcgggcggcggcggtgacggaggcgccgctgccagggggcgtgcggcagcgcggcggcgg

SEQ ID NO: 4 - DNA, 22 bp, Homo sapiens
ggctgggcctcgagcgcccgca

SEQ ID NO: 5 - DNA, 22 bp, Homo sapiens
tcgagtccctcaagtccttcca

SEQ ID NO: 6 - DNA, 22 bp, Homo sapiens
accgccatggcgaccctggaaa

SEQ ID NO: 7 - DNA, 72 bp, Homo sapiens
agaccgccatggcgaccctggaaaagctgatgaaggccttcgagtccctcaagtccttccagcagcagcagc

SEQ ID NO: 8 - DNA, 22 bp, Homo sapiens
ggagccgctgcaccgaccgtga

SEQ ID NO: 9 - DNA, 22 bp, Homo sapiens
gcaccgaccgtgagtttgggcc

SEQ ID NO: 10 - DNA, 22 bp, Homo sapiens
ccgccgcaggcacagccgctgc

SEQ ID NO: 11 - DNA, 168 bp, Homo sapiens
agcagcaacagccgccaccgccgccgccgccgccgccgcctcctcagcttcctcagccgccgccgcaggcacagccgctgctgcctcagccgcagccgcccccgccgccgcccccgccgccacccggcccggctgtggctgaggagccgctgcaccgaccgtgagttt

SEQ ID NO: 12 - DNA, 22 bp, Homo sapiens
tgggattggttgccagtgctta

SEQ ID NO: 13 - DNA, 22 bp, Homo sapiens
tcgctccgggtacgcgcgctgg

SEQ ID NO: 14 - DNA, 22 bp, Homo sapiens
cgcagagctgtgtgaccttggg

SEQ ID NO: 15 - DNA, 22 bp, Homo sapiens
tggaacgaggtgaaactttcag

SEQ ID NO: 16 - DNA, 22 bp, Homo sapiens
ccgcgggccgcacgccgcgggc

SEQ ID NO: 17 - DNA, 22 bp, Homo sapiens
tgtcctgcggtgcgactgcggg

SEQ ID NO: 18 - DNA, 22 bp, Homo sapiens
ttaggggagatgaaagaggcag

SEQ ID NO: 19 - DNA, 22 bp, Homo sapiens
ctgacccagttacgccacggct

SEQ ID NO: 20 - DNA, 22 bp, Homo sapiens
gacccagttacgccacggcttg

SEQ ID NO: 21 - DNA, 22 bp, Homo sapiens
ccgcgggccgcacgccgcacgc

SEQ ID NO: 22 - DNA, 22 bp, Homo sapiens
tgtttgcgcgcacgggcgcgcg

SEQ ID NO: 23 - DNA, 22 bp, Homo sapiens
gaagcggccttgcaactccctt

SEQ ID NO: 24 - DNA, 22 bp, Homo sapiens
aggcgccgcgcacgccggggtc

SEQ ID NO: 25 - DNA, 22 bp, Homo sapiens
gaaggtggatcacctgaggtcc

SEQ ID NO: 26 - DNA, 22 bp, Homo sapiens
taatagatggtatctgctagta

SEQ ID NO: 27 - DNA, 22 bp, Homo sapiens
agcggccttgcaactcccttct

SEQ ID NO: 28 - DNA, 22 bp, Homo sapiens
ttccgaggggtgtgcggctgtc

SEQ ID NO: 29 - DNA, 22 bp, Homo sapiens
gagggtgtttcacgaggaggga

SEQ ID NO: 30 - DNA, 22 bp, Homo sapiens
ataatgtgtgtgtctgtgtgta

SEQ ID NO: 31 - DNA, 22 bp, Homo sapiens
tgtgtgtctgtgtgtatctgta

SEQ ID NO: 32 - DNA, 22 bp, Homo sapiens
gcacgccgcacgcctgcgcagg

SEQ ID NO: 33 - DNA, 22 bp, Homo sapiens
gtgtgttgtgtgtgtgtgtttg

SEQ ID NO: 34 - DNA, 22 bp, Homo sapiens
gcggacctggtgtgaggattaa

SEQ ID NO: 35 - DNA, 22 bp, Homo sapiens
cacttctctgcgataacttgtt

SEQ ID NO: 36 - DNA, 22 bp, Homo sapiens
gtggctggtacgccgcatgtat

SEQ ID NO: 37 - DNA, 22 bp, Homo sapiens
tgctagtatatacatacacata

SEQ ID NO: 38 - DNA, 22 bp, Homo sapiens
gcgggccgcacgccgcacgcct

SEQ ID NO: 39 - DNA, 22 bp, Homo sapiens
gcgccgcgcacgccggggtcgc

SEQ ID NO: 40 - DNA, 22 bp, Homo sapiens
ggcgcgcgcacacctaatattt

SEQ ID NO: 41 - DNA, 22 bp, Homo sapiens
tgtgtgtgtttgcgcgcacggg

SEQ ID NO: 42 - DNA, 22 bp, Homo sapiens
acacataatgtgtgtgtctgtg

SEQ ID NO: 43 - DNA, 22 bp, Homo sapiens
ccacacgtgttatttggcccac

SEQ ID NO: 44 - DNA, 22 bp, Homo sapiens
ataaaggtgacgcccattttgc

SEQ ID NO: 45 - DNA, 22 bp, Homo sapiens
atgagggtcttgaagatgccaa

SEQ ID NO: 46 - DNA, 22 bp, Homo sapiens
tgccagtgcttaaaagttagga

SEQ ID NO: 47 - DNA, 22 bp, Homo sapiens
gcgtgtgtgttgtgtgtgtgtg

SEQ ID NO: 48 - DNA, 22 bp, Homo sapiens
gtgtgtgttgtgtgtgtgtgtt

SEQ ID NO: 49 - DNA, 22 bp, Homo sapiens
cgccacggcttgaaaggaggaa

SEQ ID NO: 50 - DNA, 22 bp, Homo sapiens
taaatgggaataacatagataa

SEQ ID NO: 51 - DNA, 22 bp, Homo sapiens
aggcaggccacgtccaagccat

SEQ ID NO: 52 - DNA, 22 bp, Homo sapiens
cgcggtggctcatgcccataat

SEQ ID NO: 53 - DNA, 22 bp, Homo sapiens
tgcgataacttgtttcagtaat

SEQ ID NO: 54 - DNA, 22 bp, Homo sapiens
tatctgctagtatatacataca

SEQ ID NO: 55 - DNA, 22 bp, Homo sapiens
tatatacatacacataatgtgt

SEQ ID NO: 56 - DNA, 22 bp, Homo sapiens
aaggcacgggcgaaggcagggc

SEQ ID NO: 57 - DNA, 22 bp, Homo sapiens
ctgtatatagcgtgtgtgttgt

SEQ ID NO: 58 - DNA, 22 bp, Homo sapiens
gtgttgtgtgtgtgtgtttgcg

SEQ ID NO: 59 - DNA, 22 bp, Homo sapiens
ataacatagataaagtcttcag

SEQ ID NO: 60 - DNA, 22 bp, Homo sapiens
gaagattcctcaaggggaggac

SEQ ID NO: 61 - DNA, 22 bp, Homo sapiens
gtacgccgcatgtattagggga

SEQ ID NO: 62 - DNA, 22 bp, Homo sapiens
tgtctgtgtgtatctgtatata

SEQ ID NO: 63 - DNA, 22 bp, Homo sapiens
gaacttcccacacgtgttattt

SEQ ID NO: 64 - DNA, 22 bp, Homo sapiens
tgtatctgtatatagcgtgtgt

SEQ ID NO: 65 - DNA, 22 bp, Homo sapiens
tggatttttttgaacgaaatgc

SEQ ID NO: 66 - DNA, 22 bp, Homo sapiens
acttcccacacgtgttatttgg

SEQ ID NO: 67 - DNA, 22 bp, Homo sapiens
acatggtatttaatgagggtct

SEQ ID NO: 68 - DNA, 22 bp, Homo sapiens
cggtggctcatgcccataatct

SEQ ID NO: 69 - DNA, 22 bp, Homo sapiens
tctccatgcttgtcacttctct

SEQ ID NO: 70 - DNA, 22 bp, Homo sapiens
gctgtctccatgcttgtcactt

SEQ ID NO: 71 - DNA, 22 bp, Homo sapiens
ggacctggtgtgaggattaaat

SEQ ID NO: 72 - DNA, 22 bp, Homo sapiens
gggtgtttcacgaggagggaac

SEQ ID NO: 73 - DNA, 22 bp, Homo sapiens
ctagtatatacatacacataat

SEQ ID NO: 74 - DNA, 1352 bp, Homo sapiens
ccgcgcagtaagtatccgcgccgggaacagccgcgggccgcacgccgcgggccgcacgccgcacgcctgcgcagggaggcgccgcgcacgccggggtcgctccgggtacgcgcgctggactagctcaccccgctccttctcagggcggcccggcggaagcggccttgcaactcccttctctggttctcccggttgcatttacactggcttctgctttccgaaggaaaaggggacattttgtcctgcggtgcgactgcgggtcaaggcacgggcgaaggcagggcaggctggtggaggggaccggttccgaggggtgtgcggctgtctccatgcttgtcacttctctgcgataacttgtttcagtaatattaatagatggtatctgctagtatatacatacacataatgtgtgtgtctgtgtgtatctgtatatagcgtgtgtgttgtgtgtgtgtgtttgcgcgcacgggcgcgcgcacacctaatattttcaaggctggatttttttgaacgaaatgctttcctggaacgaggtgaaactttcagagctgcagaatagctagagcagcaggggccctggcttttggaaactgacccgacctttattccagattctgccccactccgcagagctgtgtgaccttgggggattcccctaacctctctgagacgtggctttgttttctgtagggagaagataaaggtgacgcccattttgcggacctggtgtgaggattaaatgggaataacatagataaagtcttcagaacttcaaattagttcccctttcttcctttggggggtacaaagaaatatctgacccagttacgccacggcttgaaaggaggaaacccaaagaatggctgtggggatgaggaagattcctcaaggggaggacatggtatttaatgagggtcttgaagatgccaaggaagtggtagagggtgtttcacgaggagggaaccgtctgggcaaaggccaggaaggcggaaggggatcccttcagagtggctggtacgccgcatgtattaggggagatgaaagaggcaggccacgtccaagccatatttgtgttgctctccggagtttgtactttaggcttgaacttcccacacgtgttatttggcccacattgtgtttgaagaaactttgggattggttgccagtgcttaaaagttaggacttagaaaatggatttcctggcaggacgcggtggctcatgcccataatctcagcactttgggaggcctaggaaggtggatcacctgaggtccggagttcaagactaacctggccaacatggtgaaacccagtatctactaaaaaatacaaaaaaaaaaaaaaaagaagaa

SEQ ID NO: 75 - DNA, 22 bp, Homo sapiens
cgcgcgcctgtaatcccagcta

SEQ ID NO: 76 - DNA, 22 bp, Homo sapiens
caacctcaggtgatccgcccac

SEQ ID NO: 77 - DNA, 22 bp, Homo sapiens
ggcgtggtgtcgcgcgcctgta

SEQ ID NO: 78 - DNA, 22 bp, Homo sapiens
tatactgaattaatcacatttg

SEQ ID NO: 79 - DNA, 22 bp, Homo sapiens
gagaatcgcttgagcccgggag

SEQ ID NO: 80 - DNA, 22 bp, Homo sapiens
aggaggtggacactgggtttct

SEQ ID NO: 81 - DNA, 22 bp, Homo sapiens
attacaggcgtgagccaccgcg

SEQ ID NO: 82 - DNA, 22 bp, Homo sapiens
agacatttattacttggcttct

SEQ ID NO: 83 - DNA, 22 bp, Homo sapiens
gaaaaataggcaagtgtggcca

SEQ ID NO: 84 - DNA, 22 bp, Homo sapiens
taagggctattgactgacaaac

SEQ ID NO: 85 - DNA, 22 bp, Homo sapiens
agctgccacgtattgggcttcc

SEQ ID NO: 86 - DNA, 22 bp, Homo sapiens
ttttagatggtacctggtggct

SEQ ID NO: 87 - DNA, 22 bp, Homo sapiens
tttgtttttttgagacagagtt

SEQ ID NO: 88 - DNA, 22 bp, Homo sapiens
tagctgggattatcggctaatt

SEQ ID NO: 89 - DNA, 22 bp, Homo sapiens
cccctgcctgtgtggacagcat

SEQ ID NO: 90 - DNA, 22 bp, Homo sapiens
gactccgtctcaaaaaataata

SEQ ID NO: 91 - DNA, 22 bp, Homo sapiens
gaattacaggcgtgagccaccg

SEQ ID NO: 92 - DNA, 22 bp, Homo sapiens
tattgactgacaaacacaccca

SEQ ID NO: 93 - DNA, 22 bp, Homo sapiens
ggaaagcagacatttattactt

SEQ ID NO: 94 - DNA, 22 bp, Homo sapiens
gaggttgcattaagccaagatc

SEQ ID NO: 95 - DNA, 22 bp, Homo sapiens
agcagacatttattacttggct

SEQ ID NO: 96 - DNA, 1000 bp, Homo sapiens
agaaaataaagaaaagttagccgggcgtggtgtcgcgcgcctgtaatcccagctactccagaggctgcggcaggagaatcgcttgagcccgggaggcagaggttgcattaagccaagatcgcccaatgcactccggcctgggcgacagagcaagactccgtctcaaaaaataataataataaataaaaataaaaaataaaatggatttcccagcatctctggaaaaataggcaagtgtggccatgatggtccttagatctcctctaggaaagcagacatttattacttggcttctgtgcactatctgagctgccacgtattgggcttccacccctgcctgtgtggacagcatgggttgtcagcagagttgtgttttgttttgtttttttgagacagagtttccctcttgttgcccaggctggagtgcagtggctcagtctcagctcactgcaacctctgcctcctgggttcaagtgattctcctgcctcagcctcccgagtagctgggattatcggctaattttgtatttttagtagagacagatttctccatgttggtcaggctggtctcgaactcccaacctcaggtgatccgcccacctcgccctcccaaagtgctggaattacaggcgtgagccaccgcgtctggccatcagcagagtttttaatttaggagaatgacaagaggtggtacagttttttagatggtacctggtggctgttaagggctattgactgacaaacacacccaacttggcgctgccgcccaggaggtggacactgggtttctggatagatggttagcaacctctgtcaccagctgggcctctttttttctatactgaattaatcacatttgtttaacctgtctgttccatagttcccttgcacatcttgggtatttgaggagttgggtgggtggcagtggcaactggggccaccatcctgtttaattattttaaagccctgactgtcctggattgaccctaagctccccctg

SEQ ID NO: 97 - DNA, 22 bp, Homo sapiens
tgccagttcacaaccgctccga

SEQ ID NO: 98 - DNA, 22 bp, Homo sapiens
gaagactgagtgcccggggcac

SEQ ID NO: 99 - DNA, 22 bp, Homo sapiens
tccagtcctgtgatccgggccc

SEQ ID NO: 100 - DNA, 22 bp, Homo sapiens
ccgctccgagcgtgggtctccg

SEQ ID NO: 101 - DNA, 22 bp, Homo sapiens
gaactgtcttcgactccggggc

SEQ ID NO: 102 - DNA, 249 bp, Homo sapiens
gcgctccctgaaccctagaactgtcttcgactccggggccccgttggaagactgagtgcccggggcacggcacagaagccgcgcccaccgcctgccagttcacaaccgctccgagcgtgggtctccgcccagctccagtcctgtgatccgggcccgccccctagcggccggggagggaggggccgggtccgcggccggcgaacggggctcgaagggtccttgtagccgggaatgctgctgctgctgctg

SEQ ID NO: 103 - DNA, 22 bp, Homo sapiens
tagcgggatgcgaagcggccga

SEQ ID NO: 104 - DNA, 22 bp, Homo sapiens
tgcgcctgcgcacgccacgcgc

SEQ ID NO: 105 - DNA, 22 bp, Homo sapiens
ctttcttgtgcatgacgccctg

SEQ ID NO: 106 - DNA, 22 bp, Homo sapiens
ctggggggatcacagaccattt

SEQ ID NO: 107 - DNA, 22 bp, Homo sapiens
ctctggggagcgtctggcgcga

SEQ ID NO: 108 - DNA, 22 bp, Homo sapiens
gggaaggcagcaagccgggccg

SEQ ID NO: 109 - DNA, 22 bp, Homo sapiens
acgccacgcgcatccgctcctg

SEQ ID NO: 110 - DNA, 22 bp, Homo sapiens
gggccgtccgtgttccatcctc

SEQ ID NO: 111 - DNA, 22 bp, Homo sapiens
gctcctgggacgcaagctcgag

SEQ ID NO: 112 - DNA, 22 bp, Homo sapiens
tccggaggcgtgtggaggcggc

SEQ ID NO: 113 - DNA, 22 bp, Homo sapiens
ggcccagctgtgccaccgagcg

SEQ ID NO: 114 - DNA, 22 bp, Homo sapiens
ccccacctatcgttggttcgca

SEQ ID NO: 115 - DNA, 22 bp, Homo sapiens
atcgttggttcgcaaagtgcaa

SEQ ID NO: 116 - DNA, 22 bp, Homo sapiens
ggggctttggcgtccggccaat

SEQ ID NO: 117 - DNA, 22 bp, Homo sapiens
cggtatttattgtctgtcccca

SEQ ID NO: 118 - DNA, 22 bp, Homo sapiens
cgcctgcgcacgccacgcgcat

SEQ ID NO: 119 - DNA, 22 bp, Homo sapiens
cggtttgcgttgtgggccggag

SEQ ID NO: 120 - DNA, 22 bp, Homo sapiens
aatccggaggcgtgtggaggcg

SEQ ID NO: 121 - DNA, 22 bp, Homo sapiens
gaggccctgacgtggatgggca

SEQ ID NO: 122 - DNA, 22 bp, Homo sapiens
ccgaccctcgcgaataaaaggc

SEQ ID NO: 123 - DNA, 22 bp, Homo sapiens
agctttcttgtgcatgacgccc

SEQ ID NO: 124 - DNA, 22 bp, Homo sapiens
tctgcctgcttactcgggaaat

SEQ ID NO: 125 - DNA, 22 bp, Homo sapiens
tttggatatttattgacctcgt

SEQ ID NO: 126 - DNA, 22 bp, Homo sapiens
tcctccgactcgctgacaggct

SEQ ID NO: 127 - DNA, 22 bp, Homo sapiens
aatttgcttttgccaaacccgc

SEQ ID NO: 128 - DNA, 22 bp, Homo sapiens
aaagctttcttgtgcatgacgc

SEQ ID NO: 129 - DNA, 22 bp, Homo sapiens
gttttggatgcactgagacccc

SEQ ID NO: 130 - DNA, 22 bp, Homo sapiens
ccccgaccctcgcgaataaaag

SEQ ID NO: 131 - DNA, 22 bp, Homo sapiens
gcggtttggatatttattgacc

SEQ ID NO: 132 - DNA, 988 bp, Homo sapiens
gctgctgctggggggatcacagaccatttctttctttcggccaggctgaggccctgacgtggatgggcaaactgcaggcctgggaaggcagcaagccgggccgtccgtgttccatcctccacgcacccccacctatcgttggttcgcaaagtgcaaagctttcttgtgcatgacgccctgctctggggagcgtctggcgcgatctctgcctgcttactcgggaaatttgcttttgccaaacccgctttttcggggatcccgcgcccccctcctcacttgcgctgctctcggagccccagccggctccgcccgcttcggcggtttggatatttattgacctcgtcctccgactcgctgacaggctacaggacccccaacaaccccaatccacgttttggatgcactgagaccccgacattcctcggtatttattgtctgtccccacctaggacccccacccccgaccctcgcgaataaaaggccctccatctgcccaaagctctggactccacagtgtccgcggtttgcgttgtgggccggaggctccgcagcgggccaatccggaggcgtgtggaggcggccgaaggtctgggaggagctagcgggatgcgaagcggccgaatcagggttgggggaggaaaagccacggggcggggctttggcgtccggccaataggagggcgagcgggccacccggaggcaccgcccccgcccagctgtggcccagctgtgccaccgagcgtcgagaagagggggctgggctggcagcgcgcgcggccatcctccttccactgcgcctgcgcacgccacgcgcatccgctcctgggacgcaagctcgagaaaagttgctgcaaactttctagcccgttccccgcccctcctcccggccagacccgccccccctgcggagccgggaattccgaggggcggagcgcaggccgagatggggaatgtgggggcctgcagaggaccctggagacggaggcgt

SEQ ID NO: 133 - protein, 364 aa, Artificial Sequence
  Synthesized
MAPKKKRKVHMNTKYNKEFLLYLAGFVDGDGSIYATILPAQRSKFKHRLRLYFVVHQKTQRRWFLDKLVDEIGVGYVYDLGSVSEYRLSQIKPLHNFLTQLQPFLKLKQKQANLVLKIIEQLPSAKESPDKFLEVCTWVDQIAALNDSKTRKTTSETVRAVLDSLPGSVGGLSPSQASSAASSASSSPGSGISEALRAGAGSGTGYNKEFLLYLAGFVDGDGSIFARIHPEQRGKFKHELRLTFRVSQKTQRRWFLDKLVDEIGVGYVHDRGSVSDYSLSQIKPLHNFLTQLQPFLKLKQKQANLVLKIIEQLPSAKESPDKFLEVCTWVDQIAALNDSKTRKTTSETVRAVLDSLSEKKKSSP

SEQ ID NO: 134 - protein, 364 aa, Artificial Sequence
  Synthesized
MAPKKKRKVHMNTKYNKEFLLYLAGFVDGDGSIYASIMPAQHRKFKHQLHLRFAVIQKTQRRWFLDKLVDEIGVGYVSDDGSVSRYVLSQIKPLHNFLTQLQPFLKLKQKQANLVLKIIEQLPSAKESPDKFLEVCTWVDQIAALNDSKTRKTTSETVRAVLDSLPGSVGGLSPSQASSAASSASSSPGSGISEALRAGAGSGTGYNKEFLLYLAGFVDGDGSIFATIIPRQNRKFKHQLFLNFRVHQKTQRRWFLDKLVDEIGVGYVYDSGSVSIYNLSQIKPLHNFLTQLQPFLKLKQKQANLVLKIIEQLPSAKESPDKFLEVCTWVDQIAALNDSKTRKTTSETVRAVLDSLSEKKKSSP

SEQ ID NO: 135 - protein, 364 aa, Artificial Sequence
  Synthesized
MAPKKKRKVHMNTKYNKEFLLYLAGFVDGDGSIYACIRPCQTVKFKHRLLLHFMVSQKTQRRWFLDKLVDEIGVGYVQDTGSASQYRLSEIKPLHNFLTQLQPFLKLKQKQANLVLKIIEQLPSAKESPDKFLEVCTWVDQIAALNDSKTRKTTSETVRAVLDSLPGSVGGLSPSQASSAASSASSSPGSGISEALRAGAGSGTGYNKEFLLYLAGFVDGDGSIYASIIPRQWAKFKHELLLYFRVFQKTQRRWFLDKLVDEIGVGYVYDSGSVSYYHLSQIKPLHNFLTQLQPFLKLKQKQANLVLKIIEQLPSAKESPDKFLEVCTWVDQIAALNDSKTRKTTSETVRAVLDSLSEKKKSSP

SEQ ID NO: 136 - DNA, 1791 bp, Artificial Sequence
  Synthesized
cacaggtgtccactcccagttcaattacagctcttaaggctagagtacttaatacgactcactataggctagcctcgagccgccaccatggcaccgaagaagaagcgcaaggtgcatatgaatacaaaatataataaagagttcttactctacttagcagggtttgtagacggtgacggttccatctatgccactatcctgccggcgcagcgttcgaagttcaagcacaggctgaggctctatttcgtggtccatcagaagacacagcgccgttggttcctcgacaagctggtggacgaaatcggtgtgggttacgtgtatgaccttggcagcgtctccgagtaccgtctgtcccagatcaagcctttgcataattttttaacacaactacaaccttttctaaaactaaaacaaaaacaagcaaatttagttttaaaaattattgaacaacttccgtcagcaaaagaatccccggacaaattcttagaagtttgtacatgggtggatcaaattgcagctctgaatgattcgaagacgcgtaaaacaacttctgaaaccgttcgtgctgtgctagacagtttaccaggatccgtgggaggtctatcgccatctcaggcatccagcgccgcatcctcggcttcctcaagcccgggttcagggatctccgaagcactcagagctggagcaggttccggcactggatacaacaaggaattcctgctctacctggcgggcttcgtcgacggggacggctccatctttgcccgtatccatccggagcagcgtggtaagttcaagcacgagctgcgcctcaccttccgtgtcagtcagaagacacagcgccgttggttcctcgacaagctggtggacgagatcggtgtgggttacgtgcatgaccggggcagcgtctccgattactcgctgtcccagatcaagcctctgcacaacttcctgacccagctccagcccttcctgaagctcaagcagaagcaggccaacctcgtgctgaagatcatcgagcagctgccctccgccaaggaatccccggacaagttcctggaggtgtgcacctgggtggaccagatcgccgctctgaacgactccaagacccgcaagaccacttccgaaaccgtccgcgccgttctagacagtctctccgagaagaagaagtcgtccccctaaacagtctctccgagaagaagaagtcgtccccctagcggccgcttcgagcagacatgataagatacattgatgagtttggacaaaccacaactagaatgcagtgaaaaaaatgctttatttgtgaaatttgtgatgctattgctttatttgtaaccattataagctgcaataaacaagttaacaacaacaattgcattcattttatgtttcaggttcagggggagatgtgggaggttttttaaagcaagtaaaacctctacaaatgtggtaaaatcgataagatcttgatccgggctggcgtaatagcgaagaggcccgcaccgatcgcccttcccaacagttgcgcagcctgaatggcgaatggacgcgccctgtagcggcgcattaagcgcggcgggtgtggtggttacgcgcagcgtgaccgctacacttgccagcgccctagcgcccgctcctttcgctttcttcccttcctttctcgccacgttcgccggctttccccgtcaagctctaaatcgggggctccctttagggttccgatttagtgctttacggcacctcgaccccaaaaaacttgattagggtgatggttcacgtagtgggccatcg

SEQ ID NO: 137 - DNA, 1791 bp, Artificial Sequence
  Synthesized
cacaggtgtccactcccagttcaattacagctcttaaggctagagtacttaatacgactcactataggctagcctcgagccgccaccatggcaccgaagaagaagcgcaaggtgcatatgaatacaaaatataataaagagttcttactctacttagcagggtttgtagacggtgacggttccatctatgcctcgatcatgcctgcgcaacatcgtaagttcaagcaccagctgcatctccgtttcgcggtcattcagaagacacagcgccgttggttcctcgacaagctggtggacgagatcggtgtgggttacgtgtctgacgatggcagcgtctcccgttacgtgctgtcccagatcaagcctttgcataattttttaacacaactacaaccttttctaaaactaaaacaaaaacaagcaaatttagttttaaaaattattgaacaacttccgtcagcaaaagaatccccggacaaattcttagaagtttgtacatgggtggatcaaattgcagctctgaatgattcgaagacgcgtaaaacaacttctgaaaccgttcgtgctgtgctagacagtttaccaggatccgtgggaggtctatcgccatctcaggcatccagcgccgcatcctcggcttcctcaagcccgggttcagggatctccgaagcactcagagctggagcaggttccggcactggatacaacaaggaattcctgctctacctggcgggcttcgtcgacggggacggctccatctttgccactatcattcctaggcaaaatcggaagttcaagcaccagctgtttctcaatttccgtgtccatcagaagacacagcgccgttggttcctcgacaagctggtggacgagatcggtgtgggttacgtgtatgactctggcagcgtctccatttacaatctgtcccagatcaagcctctgcacaacttcctgacccagctccagcccttcctgaagctcaagcagaagcaggccaacctcgtgctgaagatcatcgagcagctgccctccgccaaggaatccccggacaagttcctggaggtgtgcacctgggtggaccagatcgccgctctgaacgactccaagacccgcaagaccacttccgaaaccgtccgcgccgttctagacagtctctccgagaagaagaagtcgtccccctaaacagtctctccgagaagaagaagtcgtccccctagcggccgcttcgagcagacatgataagatacattgatgagtttggacaaaccacaactagaatgcagtgaaaaaaatgctttatttgtgaaatttgtgatgctattgctttatttgtaaccattataagctgcaataaacaagttaacaacaacaattgcattcattttatgtttcaggttcagggggagatgtgggaggttttttaaagcaagtaaaacctctacaaatgtggtaaaatcgataagatcttgatccgggctggcgtaatagcgaagaggcccgcaccgatcgcccttcccaacagttgcgcagcctgaatggcgaatggacgcgccctgtagcggcgcattaagcgcggcgggtgtggtggttacgcgcagcgtgaccgctacacttgccagcgccctagcgcccgctcctttcgctttcttcccttcctttctcgccacgttcgccggctttccccgtcaagctctaaatcgggggctccctttagggttccgatttagtgctttacggcacctcgaccccaaaaaacttgattagggtgatggttcacgtagtgggccatcg

SEQ ID NO: 138 - DNA, 1791 bp, Artificial Sequence
  Synthesized
cacaggtgtccactcccagttcaattacagctcttaaggctagagtacttaatacgactcactataggctagcctcgagccgccaccatggcaccgaagaagaagcgcaaggtgcatatgaatacaaaatataataaagagttcttactctacttagcagggtttgtagacggtgacggttccatctatgcctgtatccggccttgtcaaacggtgaagttcaagcaccgtctgctgctccatttcatggtcagtcagaagacacagcgccgttggttcctcgacaagctggtggacgagatcggtgtgggttacgtgcaggacactggcagcgcctcccagtaccggctgtccgagatcaagcctttgcataattttttaacacaactacaaccttttctaaaactaaaacaaaaacaagcaaatttagttttaaaaattattgaacaacttccgtcagcaaaagaatccccggacaaattcttagaagtttgtacatgggtggatcaaattgcagctctgaatgattcgaagacgcgtaaaacaacttctgaaaccgttcgtgctgtgctagacagtttaccaggatccgtgggaggtctatcgccatctcaggcatccagcgccgcatcctcggcttcctcaagcccgggttcagggatctccgaagcactcagagctggagcaggttccggcactggatacaacaaggaattcctgctctacctggcgggcttcgtcgacggggacggctccatctatgcctctatcattcctcgtcaatgggctaagttcaagcacgagctgcttctctatttccgtgtctttcagaagacacagcgccgttggttcctcgacaagctggtggacgagatcggtgtgggttacgtgtatgacagtggcagcgtctcctattaccatctgtcccagatcaagcctctgcacaacttcctgacccagctccagcccttcctgaagctcaagcagaagcaggccaacctcgtgctgaagatcatcgagcagctgccctccgccaaggaatccccggacaagttcctggaggtgtgcacctgggtggaccagatcgccgctctgaacgactccaagacccgcaagaccacttccgaaaccgtccgcgccgttctagacagtctctccgagaagaagaagtcgtccccctaaacagtctctccgagaagaagaagtcgtccccctagcggccgcttcgagcagacatgataagatacattgatgagtttggacaaaccacaactagaatgcagtgaaaaaaatgctttatttgtgaaatttgtgatgctattgctttatttgtaaccattataagctgcaataaacaagttaacaacaacaattgcattcattttatgtttcaggttcagggggagatgtgggaggttttttaaagcaagtaaaacctctacaaatgtggtaaaatcgataagatcttgatccgggctggcgtaatagcgaagaggcccgcaccgatcgcccttcccaacagttgcgcagcctgaatggcgaatggacgcgccctgtagcggcgcattaagcgcggcgggtgtggtggttacgcgcagcgtgaccgctacacttgccagcgccctagcgcccgctcctttcgctttcttcccttcctttctcgccacgttcgccggctttccccgtcaagctctaaatcgggggctccctttagggttccgatttagtgctttacggcacctcgaccccaaaaaacttgattagggtgatggttcacgtagtgggccatcg

SEQ ID NO: 139 - DNA, 23 bp, Artificial Sequence
  Synthesized
ccagttacgccacggcttgaaag

SEQ ID NO: 140 - DNA, 24 bp, Artificial Sequence
  Synthesized
ctctgctgacaacccatgctgtcc

SEQ ID NO: 141 - DNA, 22 bp, Homo sapiens
tgaaggccttcgagtccctcaa

SEQ ID NO: 142 - DNA, 90 bp, Homo sapiens
gcggcggcggctgggcctcgagcgcccgcagcccacctctcgggggcgggctcccggcgctagcagggctgaagagaagatggaggagct

SEQ ID NO: 143 - protein, 354 aa, Artificial Sequence
  Synthesized
MNTKYNKEFLLYLAGFVDGDGSIYATILPAQRSKFKHRLRLYFVVHQKTQRRWFLDKLVDEIGVGYVYDLGSVSEYRLSQIKPLHNFLTQLQPFLKLKQKQANLVLKIIEQLPSAKESPDKFLEVCTWVDQIAALNDSKTRKTTSETVRAVLDSLPGSVGGLSPSQASSAASSASSSPGSGISEALRAGAGSGTGYNKEFLLYLAGFVDGDGSIFARIHPEQRGKFKHELRLTFRVSQKTQRRWFLDKLVDEIGVGYVHDRGSVSDYSLSQIKPLHNFLTQLQPFLKLKQKQANLVLKIIEQLPSAKESPDKFLEVCTWVDQIAALNDSKTRKTTSETVRAVLDSLSEKKKSSP

SEQ ID NO: 144 - protein, 354 aa, Artificial Sequence
  Synthesized
MNTKYNKEFLLYLAGFVDGDGSIYATIVPCQTGKFKHRLRLWFSVYQKTQRRWFLDKLVDEIGVGYVVDNGSVSEYRLSEIKPLHNFLTQLQPFLKLKQKQANLVLKIIEQLPSAKESPDKFLEVCTWVDQIAALNDSKTRKTTSETVRAVLDSLPGSVGGLSPSQASSAASSASSSPGSGISEALRAGAGSGTGYNKEFLLYLAGFVDGDGSIYARICPDQRAKFKHVLELRFRVTQKTQRRWFLDKLVDEIGVGYVHDRGSVSDYQLSQIKPLHNFLTQLQPFLKLKQKQANLVLKIIEQLPSAKESPDKFLEVCTWVDQIAALNDSKTRKTTSETVRAVLDSLSEKKKSSP

SEQ ID NO: 145 - protein, 354 aa, Artificial Sequence
  Synthesized
MNTKYNKEFLLYLAGFVDGDGSIYACIEPGQTGKFKHRLKLVFEVYQKTQRRWFLDKLVDEIGVGYVVGSGSVSSYRLSEIKPLHNFLTQLQPFLKLKQKQANLVLKIIEQLPSAKESPDKFLEVCTWVDQIAALNDSKTRKTTSETVRAVLDSLPGSVGGLSPSQASSAASSASSSPGSGISEALRAGAGSGTGYNKEFLLYLAGFVDGDGSIYARICPDQRAKFKHVLEPRFRVTQKTQRRWFLDKLVDEIGVGYVHDRGSVSDYQLSQIKPLHNFLTQLQPFLKLKQKQANLVLKIIEQLPSAKESPDKFLEVCTWVDQIAALNDSKTRKTTSETVRAVLDSLSEKKKSSP

SEQ ID NO: 146 - protein, 354 aa, Artificial Sequence
  Synthesized
MNTKYNKEFLLYLAGFVDGDGSIYASIFPGQNQKFKHRLRLYFAVFQKTQRRWFLDKLVDEIGVGYVYDIGSVPEYRLSQIKPLHNFLTQLQPFLKLKQKQANLVLKIIEQLPSAKESPDKFLEVCTWVDQIAALNDSKTRKTTSETVRAVLDSLPGSVGGLSPSQASSAASSASSSPGSGISEALRAGAGSGTGYNKEFLLYLAGFVDGDGSIYARICPDQRGKFKHGLELRFRVTQKTQRRWFLDKLVDEIGVGYVNDRGSVSDYHLSQIKPLHNFLTQLQPFLKLKQKQANLVLKIIEQLPSAKESPDKFLEVCTWVDQIAALNDSKTRKTTSETVRAVLDSLSEKKKSSP

SEQ ID NO: 147 - protein, 147 aa, Artificial Sequence
  Synthesized
KEFLLYLAGFVDGDGSIYATILPAQRSKFKHRLRLYFVVHQKTQRRWFLDKLVDEIGVGYVYDLGSVSEYRLSQIKPLHNFLTQLQPFLKLKQKQANLVLKIIEQLPSAKESPDKFLEVCTWVDQIAALNDSKTRKTTSETVRAVLD

SEQ ID NO: 148 - protein, 147 aa, Artificial Sequence
  Synthesized
KEFLLYLAGFVDGDGSIYATIVPCQTGKFKHRLRLWFSVYQKTQRRWFLDKLVDEIGVGYVVDNGSVSEYRLSEIKPLHNFLTQLQPFLKLKQKQANLVLKIIEQLPSAKESPDKFLEVCTWVDQIAALNDSKTRKTTSETVRAVLD

SEQ ID NO: 149 - protein, 147 aa, Artificial Sequence
  Synthesized
KEFLLYLAGFVDGDGSIYACIEPGQTGKFKHRLKLVFEVYQKTQRRWFLDKLVDEIGVGYVVGSGSVSSYRLSEIKPLHNFLTQLQPFLKLKQKQANLVLKIIEQLPSAKESPDKFLEVCTWVDQIAALNDSKTRKTTSETVRAVLD

SEQ ID NO: 150 - protein, 147 aa, Artificial Sequence
  Synthesized
KEFLLYLAGFVDGDGSIYASIFPGQNQKFKHRLRLYFAVFQKTQRRWFLDKLVDEIGVGYVYDIGSVPEYRLSQIKPLHNFLTQLQPFLKLKQKQANLVLKIIEQLPSAKESPDKFLEVCTWVDQIAALNDSKTRKTTSETVRAVLD

SEQ ID NO: 151 - protein, 147 aa, Artificial Sequence
  Synthesized
KEFLLYLAGFVDGDGSIFARIHPEQRGKFKHELRLTFRVSQKTQRRWFLDKLVDEIGVGYVHDRGSVSDYSLSQIKPLHNFLTQLQPFLKLKQKQANLVLKIIEQLPSAKESPDKFLEVCTWVDQIAALNDSKTRKTTSETVRAVLD

SEQ ID NO: 152 - protein, 147 aa, Artificial Sequence
  Synthesized
KEFLLYLAGFVDGDGSIYARICPDQRAKFKHVLELRFRVTQKTQRRWFLDKLVDEIGVGYVHDRGSVSDYQLSQIKPLHNFLTQLQPFLKLKQKQANLVLKIIEQLPSAKESPDKFLEVCTWVDQIAALNDSKTRKTTSETVRAVLD

SEQ ID NO: 153 - protein, 147 aa, Artificial Sequence
  Synthesized
KEFLLYLAGFVDGDGSIYARICPDQRAKFKHVLEPRFRVTQKTQRRWFLDKLVDEIGVGYVHDRGSVSDYQLSQIKPLHNFLTQLQPFLKLKQKQANLVLKIIEQLPSAKESPDKFLEVCTWVDQIAALNDSKTRKTTSETVRAVLD

SEQ ID NO: 154 - protein, 147 aa, Artificial Sequence
  Synthesized
KEFLLYLAGFVDGDGSIYARICPDQRGKFKHGLELRFRVTQKTQRRWFLDKLVDEIGVGYVNDRGSVSDYHLSQIKPLHNFLTQLQPFLKLKQKQANLVLKIIEQLPSAKESPDKFLEVCTWVDQIAALNDSKTRKTTSETVRAVLD

SEQ ID NO: 155 - protein, 354 aa, Artificial Sequence
  Synthesized
MNTKYNKEFLLYLAGFVDGDGSIFALIDPRQASKFKHGLRLRFRVYQKTQRRWFLDKLVDEIGVGYVCDNGSMSAYTLSEIKPLHNFLTQLQPFLKLKQKQANLVLKIIEQLPSAKESPDKFLEVCTWVDQIAALNDSKTRKTTSETVRAVLDSLPGSVGGLSPSQASSAASSASSSPGSGISEALRAGAGSGTGYNKEFLLYLAGFVDGDGSIYARIVPMQEAKFKHVLQLRFQVTQKTQRRWFLDKLVDEIGVGYVYDRGGASDYRLSEIKPLHNFLTQLQPFLKLKQKQANLVLKIIEQLPSAKESPDKFLEVCTWVDQIAALNDSKTRKTTSETVRAVLDSLSEKKKSSP

SEQ ID NO: 156 - protein, 354 aa, Artificial Sequence
  Synthesized
MNTKYNKEFLLYLAGFVDGDGSIFALIDPRQASKFKHGLRLRFRVYQKTQRRWFLDKLVDEIGVGYVCDSGSMSTYTLSEIKPLHNFLTQLQPFLKLKQKQANLVLKIIEQLPSAKESPDKFLEVCTWVDQIAALNDSKTRKTTSETVRAVLDSLPGSVGGLSPSQASSAASSASSSPGSGISEALRAGAGSGTGYNKEFLLYLAGFVDGDGSIYARIVPMQEAKFKHVLQLRFQVTQKTQRRWFLDKLVDEIGVGYVYDRGGASDYRLSEIKPLHNFLTQLQPFLKLKQKQANLVLKIIEQLPSAKESPDKFLEVCTWVDQIAALNDSKTRKTTSETVRAVLDSLSEKKKSSP

SEQ ID NO: 157 - protein, 354 aa, Artificial Sequence
  Synthesized
MNTKYNKEFLLYLAGFVDGDGSIFALIDPRQASKFKHGLRLRFRVYQKTQRRWFLDKLVDEIGVGYVCDCGSNSQYTLSEIKPLHNFLTQLQPFLKLKQKQANLVLKIIEQLPSAKESPDKFLEVCTWVDQIAALNDSKTRKTTSETVRAVLDSLPGSVGGLSPSQASSAASSASSSPGSGISEALRAGAGSGTGYNKEFLLYLAGFVDGDGSIYARIVPMQEAKFKHVLQLRFQVTQKTQRRWFLDKLVDEIGVGYVYDRGGASDYRLSEIKPLHNFLTQLQPFLKLKQKQANLVLKIIEQLPSAKESPDKFLEVCTWVDQIAALNDSKTRKTTSETVRAVLDSLSEKKKSSP

SEQ ID NO: 158 - protein, 354 aa, Artificial Sequence
  Synthesized
MNTKYNKEFLLYLAGFVDGDGSIFALIDPRQASKFKHGLRLRFRVYQKTQRRWFLDKLVDEIGVGYVCDSGSVSQYTLSEIKPLHNFLTQLQPFLKLKQKQANLVLKIIEQLPSAKESPDKFLEVCTWVDQIAALNDSKTRKTTSETVRAVLDSLPGSVGGLSPSQASSAASSASSSPGSGISEALRAGAGSGTGYNKEFLLYLAGFVDGDGSIYARIVPMQGGKFKHSLQLKFQVTQKTQRRWFLDKLVDEIGVGYVPDRGSVSDYRLSEIKPLHNFLTQLQPFLKLKQKQANLVLKIIEQLPSAKESPDKFLEVCTWVDQIAALNDSKTRKTTSETVRAVLDSLSEKKKSSP

SEQ ID NO: 159 - protein, 354 aa, Artificial Sequence
  Synthesized
MNTKYNKEFLLYLAGFVDGDGSIYACINPGQSGKFKHRLLLRFRVSQKTQRRWFLDKLVDEIGVGYVSDSGSVSEYTLSQIKPLHNFLTQLQPFLKLKQKQANLVLKIIEQLPSAKESPDKFLEVCTWVDQIAALNDSKTRKTTSETVRAVLDSLPGSVGGLSPSQASSAASSASSSPGSGISEALRAGAGSGTGYNKEFLLYLAGFVDGDGSIYARIAPHQGMKFKHQLQLVFRVTQKTQRRWFLDKLVDEIGVGYVHDRGGASDYSLSQIKPLHNFLTQLQPFLKLKQKQANLVLKIIEQLPSAKESPDKFLEVCTWVDQIAALNDSKTRKTTSETVRAVLDSLSEKKKSSP

SEQ ID NO: 160 - protein, 147 aa, Artificial Sequence
  Synthesized
KEFLLYLAGFVDGDGSIFALIDPRQASKFKHGLRLRFRVYQKTQRRWFLDKLVDEIGVGYVCDNGSMSAYTLSEIKPLHNFLTQLQPFLKLKQKQANLVLKIIEQLPSAKESPDKFLEVCTWVDQIAALNDSKTRKTTSETVRAVLD

SEQ ID NO: 161 - protein, 147 aa, Artificial Sequence
  Synthesized
KEFLLYLAGFVDGDGSIFALIDPRQASKFKHGLRLRFRVYQKTQRRWFLDKLVDEIGVGYVCDSGSMSTYTLSEIKPLHNFLTQLQPFLKLKQKQANLVLKIIEQLPSAKESPDKFLEVCTWVDQIAALNDSKTRKTTSETVRAVLD

SEQ ID NO: 162 - protein, 147 aa, Artificial Sequence
  Synthesized
KEFLLYLAGFVDGDGSIFALIDPRQASKFKHGLRLRFRVYQKTQRRWFLDKLVDEIGVGYVCDCGSNSQYTLSEIKPLHNFLTQLQPFLKLKQKQANLVLKIIEQLPSAKESPDKFLEVCTWVDQIAALNDSKTRKTTSETVRAVLD

SEQ ID NO: 163 - protein, 147 aa, Artificial Sequence
  Synthesized
KEFLLYLAGFVDGDGSIFALIDPRQASKFKHGLRLRFRVYQKTQRRWFLDKLVDEIGVGYVCDSGSVSQYTLSEIKPLHNFLTQLQPFLKLKQKQANLVLKIIEQLPSAKESPDKFLEVCTWVDQIAALNDSKTRKTTSETVRAVLD

SEQ ID NO: 164 - protein, 147 aa, Artificial Sequence
  Synthesized
KEFLLYLAGFVDGDGSIYACINPGQSGKFKHRLLLRFRVSQKTQRRWFLDKLVDEIGVGYVSDSGSVSEYTLSQIKPLHNFLTQLQPFLKLKQKQANLVLKIIEQLPSAKESPDKFLEVCTWVDQIAALNDSKTRKTTSETVRAVLD

SEQ ID NO: 165 - protein, 147 aa, Artificial Sequence
  Synthesized
KEFLLYLAGFVDGDGSIYARIVPMQEAKFKHVLQLRFQVTQKTQRRWFLDKLVDEIGVGYVYDRGGASDYRLSEIKPLHNFLTQLQPFLKLKQKQANLVLKIIEQLPSAKESPDKFLEVCTWVDQIAALNDSKTRKTTSETVRAVLD

SEQ ID NO: 166 - protein, 147 aa, Artificial Sequence; identical to SEQ ID NO: 165
  Synthesized

SEQ ID NO: 167 - protein, 147 aa, Artificial Sequence; identical to SEQ ID NO: 165
  Synthesized

SEQ ID NO: 168 - protein, 147 aa, Artificial Sequence
  Synthesized
KEFLLYLAGFVDGDGSIYARIVPMQGGKFKHSLQLKFQVTQKTQRRWFLDKLVDEIGVGYVPDRGSVSDYRLSEIKPLHNFLTQLQPFLKLKQKQANLVLKIIEQLPSAKESPDKFLEVCTWVDQIAALNDSKTRKTTSETVRAVLD

SEQ ID NO: 169 - protein, 147 aa, Artificial Sequence
  Synthesized
KEFLLYLAGFVDGDGSIYARIAPHQGMKFKHQLQLVFRVTQKTQRRWFLDKLVDEIGVGYVHDRGGASDYSLSQIKPLHNFLTQLQPFLKLKQKQANLVLKIIEQLPSAKESPDKFLEVCTWVDQIAALNDSKTRKTTSETVRAVLD

SEQ ID NO: 170 - protein, 354 aa, Artificial Sequence
  Synthesized
MNTKYNKEFLLYLAGFVDGDGSIFACIRPSQTSKFKHRLLLHFMVSQKTQRRWFLDKLVDEIGVGYVQDMGSASQYRLSEIKPLHNFLTQLQPFLKLKQKQANLVLKIIEQLPSAKESPDKFLEVCTWVDQIAALNDSKTRKTTSETVRAVLDSLPGSVGGLSPSQASSAASSASSSPGSGISEALRAGAGSGTGYNKEFLLYLAGFVDGDGSIYASIIPRQWAKFKHELLLYFRVFQKTQRRWFLDKLVDEIGVGYVYDSGSVSYYHLSQIKPLHNFLTQLQPFLKLKQKQANLVLKIIEQLPSAKESPDKFLEVCTWVDQIAALNDSKTRKTTSETVRAVLDSLSEKKKSSP

SEQ ID NO: 171 - protein, 354 aa, Artificial Sequence
  Synthesized
MNTKYNKEFLLYLAGFVDGDGSIFACIRPSQSCKFKHRLLLHFMVCQKTQRRWFLDKLVDEIGVGYVQDTGSASQYRLSEIKPLHNFLTQLQPFLKLKQKQANLVLKIIEQLPSAKESPDKFLEVCTWVDQIAALNDSKTRKTTSETVRAVLDSLPGSVGGLSPSQASSAASSASSSPGSGISEALRAGAGSGTGYNKEFLLYLAGFVDGDGSIYASIIPRQWAKFKHELLLYFRVFQKTQRRWFLDKLVDEIGVGYVYDSGSVSYYHLSQIKPLHNFLTQLQPFLKLKQKQANLVLKIIEQLPSAKESPDKFLEVCTWVDQIAALNDSKTRKTTSETVRAVLDSLSEKKKSSP

SEQ ID NO: 172 - protein, 354 aa, Artificial Sequence
  Synthesized
MNTKYNKEFLLYLAGFVDGDGSIYACIRPCQTVKFKHRLLLHFMVSQKTQRRWFLDKLVDEIGVGYVQDTGSASQYRLSEIKPLHNFLTQLQPFLKLKQKQANLVLKIIEQLPSAKESPDKFLEVCTWVDQIAALNDSKTRKTTSETVRAVLDSLPGSVGGLSPSQASSAASSASSSPGSGISEALRAGAGSGTGYNKEFLLYLAGFVDGDGSIYASIIPRQWAKFKHELLLYFRVFQKTQRRWFLDKLVDEIGVGYVYDSGSVSYYHLSQIKPLHNFLTQLQPFLKLKQKQANLVLKIIEQLPSAKESPDKFLEVCTWVDQIAALNDSKTRKTTSETVRAVLDSLSEKKKSSP

SEQ ID NO: 173 - protein, 354 aa, Artificial Sequence
  Synthesized
MNTKYNKEFLLYLAGFVDGDGSIYASIRPEQQAKFKHYLSLYFRVIQKTQRRWFLDELVDEIGVGYVYDSGSVSYYHLSEIKPLHNFLTQLQPFLKLKQKQANLVLKIIEQLPSAKESPDKFLEVCTWVDQIAALNDSKTRKTTSETVRAVLDSLPGSVGGLSPSQASSAASSASSSPGSGISEALRAGAGSGTGYNKEFLLYLAGFVDGDGSIFACIRPAQTLKFKHRLELWFTVTQKTQRRWLLDKLVDEIGVGYVYDDGSVSRYRLSEIKPLHNFLTQLQPFLKLKQKQANLVLKIIEQLPSAKESPDKFLEVCTWVDQIAALNDSKTRKTTSETVRAVLDSLSEKKKSSP

SEQ ID NO: 174 - protein, 147 aa, Artificial Sequence
  Synthesized
KEFLLYLAGFVDGDGSIYASIIPRQWAKFKHELLLYFRVFQKTQRRWFLDKLVDEIGVGYVYDSGSVSYYHLSQIKPLHNFLTQLQPFLKLKQKQANLVLKIIEQLPSAKESPDKFLEVCTWVDQIAALNDSKTRKTTSETVRAVLD

SEQ ID NO: 175 - protein, 147 aa, Artificial Sequence; identical to SEQ ID NO: 174
  Synthesized

SEQ ID NO: 176 - protein, 147 aa, Artificial Sequence; identical to SEQ ID NO: 174
  Synthesized

SEQ ID NO: 177 - protein, 147 aa, Artificial Sequence
  Synthesized
KEFLLYLAGFVDGDGSIYASIRPEQQAKFKHYLSLYFRVIQKTQRRWFLDELVDEIGVGYVYDSGSVSYYHLSEIKPLHNFLTQLQPFLKLKQKQANLVLKIIEQLPSAKESPDKFLEVCTWVDQIAALNDSKTRKTTSETVRAVLD

SEQ ID NO: 178 - protein, 147 aa, Artificial Sequence
  Synthesized
KEFLLYLAGFVDGDGSIFACIRPSQTSKFKHRLLLHFMVSQKTQRRWFLDKLVDEIGVGYVQDMGSASQYRLSEIKPLHNFLTQLQPFLKLKQKQANLVLKIIEQLPSAKESPDKFLEVCTWVDQIAALNDSKTRKTTSETVRAVLD

SEQ ID NO: 179 - protein, 147 aa, Artificial Sequence
  Synthesized
KEFLLYLAGFVDGDGSIFACIRPSQSCKFKHRLLLHFMVCQKTQRRWFLDKLVDEIGVGYVQDTGSASQYRLSEIKPLHNFLTQLQPFLKLKQKQANLVLKIIEQLPSAKESPDKFLEVCTWVDQIAALNDSKTRKTTSETVRAVLD

SEQ ID NO: 180 - protein, 147 aa, Artificial Sequence
  Synthesized
KEFLLYLAGFVDGDGSIYACIRPCQTVKFKHRLLLHFMVSQKTQRRWFLDKLVDEIGVGYVQDTGSASQYRLSEIKPLHNFLTQLQPFLKLKQKQANLVLKIIEQLPSAKESPDKFLEVCTWVDQIAALNDSKTRKTTSETVRAVLD

SEQ ID NO: 181 - protein, 147 aa, Artificial Sequence
  Synthesized
KEFLLYLAGFVDGDGSIFACIRPAQTLKFKHRLELWFTVTQKTQRRWLLDKLVDEIGVGYVYDDGSVSRYRLSEIKPLHNFLTQLQPFLKLKQKQANLVLKIIEQLPSAKESPDKFLEVCTWVDQIAALNDSKTRKTTSETVRAVLD

SEQ ID NO: 182 - protein, 354 aa, Artificial Sequence
  Synthesized
MNTKYNKEFLLYLAGFVDGDGSIYASIMPAQHRKFKHQLHLRFAVIQKTQRRWFLDKLVDEIGVGYVSDDGSVSRYVLSQIKPLHNFLTQLQPFLKLKQKQANLVLKIIEQLPSAKESPDKFLEVCTWVDQIAALNDSKTRKTTSETVRAVLDSLPGSVGGLSPSQASSAASSASSSPGSGISEALRAGAGSGTGYNKEFLLYLAGFVDGDGSIFATIIPRQNRKFKHQLFLNFRVHQKTQRRWFLDKLVDEIGVGYVYDSGSVSIYNLSQIKPLHNFLTQLQPFLKLKQKQANLVLKIIEQLPSAKESPDKFLEVCTWVDQIAALNDSKTRKTTSETVRAVLDSLSEKKKSSP

SEQ ID NO: 183 - protein, 354 aa, Artificial Sequence
  Synthesized
MNTKYNKEFLLYLAGFVDGDGSIFAYIQPGQSYKFKHQLHLTFAVTQKTQRRWFLDKLVDEIGVGYVRDCGSVSRYYLSQIKPLHNFLTQLQPFLKLKQKQANLVLKIIEQLPSAKESPDKFLEVCTWVDQIAALNDSKTRKTTSETVRAVLDSLPGSVGGLSPSQASSAASSASSSPGSGISEALRAGAGSGTGYNKEFLLYLAGFVDGDGSIYASIRPTQWPKFKHSLVLSFRVHQKTQRRWFLDKLVDEIGVGYVYDSGGASAYHLSQIKPLHNFLTQLQPFLKLKQKQANLVLKIIEQLPSAKESPDKFLEVCTWVDQIAALNDSKTRKTTSETVRAVLDSLSEKKKSSP

SEQ ID NO: 184 - protein, 354 aa, Artificial Sequence
  Synthesized
MNTKYNKEFLLYLAGFVDGDGSIYATIRPTQRGKFKHRLELFFKVIQKTQRRWFLDKLVDEIGVGYVYDDGSVSRYYLSEIKPLHNFLTQLQPFLKLKQKQANLVLKIIEQLPSAKESPDKFLEVCTWVDQIAALNDSKTRKTTSETVRAVLDSLPGSVGGPSPSQASSAASSASSSPGSGISEALRAGAGSGTGYNKEFLLYLAGFVDGDGSIYASISPVQTCKFKHQLHLRFDVAQKTQRRWFLDKLVDEIGVGYVQDDGSVSHYKLSQIKPLHNFLTQLQPFLKLKQKQANLVLKIIEQLPSAKESPDKFLEVCTWVDQIAALNDSKTRKTTSETVRAVLDSLSEKKKSSP

SEQ ID NO: 185 - protein, 354 aa, Artificial Sequence
  Synthesized
MNTKYNKEFLLYLAGFVDGDGSIFASIQPTQDSKFKHQLHLRFVVTQKTQRRWFLDKLVDEIGVGYVQDSGSVSRYYLSEIKPLHNFLTQLQPFLKLKQKQANLVLKIIEQLPSAKESPDKFLEVCTWVDQIAALNDSKTRKTTSETVRAVLDSLPGSVGGLSPSQASSAASSASSSPGSGISEALRAGAGSGTGYNKEFLLYLAGFVDGDGSIFASIRPLQTHKFKHTLCLVFRVHQKTQRRWFLDKLVDEIGVGYVYDSGGASMYHLSEIKPLHNFLTQLQPFLKLKQKQANLVLKIIEQLPSAKESPDKFLEVCTWVDQIAALNDSKTRKTTSETVRAVLDSLSEKKKSSP

SEQ ID NO: 186 - protein, 147 aa, Artificial Sequence
  Synthesized
KEFLLYLAGFVDGDGSIFATIIPRQNRKFKHQLFLNFRVHQKTQRRWFLDKLVDEIGVGYVYDSGSVSIYNLSQIKPLHNFLTQLQPFLKLKQKQANLVLKIIEQLPSAKESPDKFLEVCTWVDQIAALNDSKTRKTTSETVRAVLD

SEQ ID NO: 187 - protein, 147 aa, Artificial Sequence
  Synthesized
KEFLLYLAGFVDGDGSIYASIRPTQWPKFKHSLVLSFRVHQKTQRRWFLDKLVDEIGVGYVYDSGGASAYHLSQIKPLHNFLTQLQPFLKLKQKQANLVLKIIEQLPSAKESPDKFLEVCTWVDQIAALNDSKTRKTTSETVRAVLD

SEQ ID NO: 188 - protein, 147 aa, Artificial Sequence
  Synthesized
KEFLLYLAGFVDGDGSIYASISPVQTCKFKHQLHLRFDVAQKTQRRWFLDKLVDEIGVGYVQDDGSVSHYKLSQIKPLHNFLTQLQPFLKLKQKQANLVLKIIEQLPSAKESPDKFLEVCTWVDQIAALNDSKTRKTTSETVRAVLD

SEQ ID NO: 189 - protein, 147 aa, Artificial Sequence
  Synthesized
KEFLLYLAGFVDGDGSIFASIRPLQTHKFKHTLCLVFRVHQKTQRRWFLDKLVDEIGVGYVYDSGGASMYHLSEIKPLHNFLTQLQPFLKLKQKQANLVLKIIEQLPSAKESPDKFLEVCTWVDQIAALNDSKTRKTTSETVRAVLD

SEQ ID NO: 190 - protein, 147 aa, Artificial Sequence
  Synthesized
KEFLLYLAGFVDGDGSIYASIMPAQHRKFKHQLHLRFAVIQKTQRRWFLDKLVDEIGVGYVSDDGSVSRYVLSQIKPLHNFLTQLQPFLKLKQKQANLVLKIIEQLPSAKESPDKFLEVCTWVDQIAALNDSKTRKTTSETVRAVLD

SEQ ID NO: 191 - protein, 147 aa, Artificial Sequence
  Synthesized
KEFLLYLAGFVDGDGSIFAYIQPGQSYKFKHQLHLTFAVTQKTQRRWFLDKLVDEIGVGYVRDCGSVSRYYLSQIKPLHNFLTQLQPFLKLKQKQANLVLKIIEQLPSAKESPDKFLEVCTWVDQIAALNDSKTRKTTSETVRAVLD

SEQ ID NO: 192 - protein, 147 aa, Artificial Sequence
  Synthesized
KEFLLYLAGFVDGDGSIYATIRPTQRGKFKHRLELFFKVIQKTQRRWFLDKLVDEIGVGYVYDDGSVSRYYLSEIKPLHNFLTQLQPFLKLKQKQANLVLKIIEQLPSAKESPDKFLEVCTWVDQIAALNDSKTRKTTSETVRAVLD

SEQ ID NO: 193 - protein, 147 aa, Artificial Sequence
  Synthesized
KEFLLYLAGFVDGDGSIFASIQPTQDSKFKHQLHLRFVVTQKTQRRWFLDKLVDEIGVGYVQDSGSVSRYYLSEIKPLHNFLTQLQPFLKLKQKQANLVLKIIEQLPSAKESPDKFLEVCTWVDQIAALNDSKTRKTTSETVRAVLD

SEQ ID NO: 194 - DNA, 22 bp, Homo sapiens
gaaagagaggtgcgtcaaacag

SEQ ID NO: 195 - DNA, 22 bp, Homo sapiens
gcggttgcggtgcctgcgcccg

SEQ ID NO: 196 - DNA, 22 bp, Homo sapiens
cgaagctgggtgtcgggctttc

SEQ ID NO: 197 - DNA, 22 bp, Homo sapiens
gtttaggaggtgtgtgtttttg

SEQ ID NO: 198 - protein, 344 aa, Artificial Sequence
  Synthesized
MNTKYNKEFLLYLAGFVDGDGSIFAYIQPAQNSKFKHLLKLVFTVTQKTQRRWFLDKLVDEIGVGYVRDHGSVSYYTLSQIKPLHNFLTQLQPFLKLKQKQANLVLKIIEQLPSAKESPDKFLEVCTWVDQIAALNDSKTRKTTSETVRAVLDSLPGSVGGLSPSQASSAASSASSSPGSGISEALRAGAGSGTGYNKEFLLYLAGFVDGDGSIYAQITPTQGLKFKHRLSLWFNVTQKTQRRWFLDKLVDEIGVGYVYDSGSVSRYILSQIKPLHNFLTQLQPFLKLKQKQANLVLKIIEQLPSAKESPDKFLEVCTWVDQIAALNDSKTRKTTSETVRAVLD

SEQ ID NO: 199 - protein, 344 aa, Artificial Sequence
  Synthesized
MNTKYNKEFLLYLAGFVDGDGSIFAYIQPAQNSKFKHLLKLVFTVTQKTQRRWFLDKLADEIGVGYVRDAGSVSYYTLSQIKPLHNFLTQLQPFLKLKQKQANLVLKIIEQLPSAKESPDKFLEVCTWVDQIAALNDSKTRKTTSETVRAVLDSLPGSVGGLSPSQASSAASSASSSPGSGISEALRAGAGSGTGYNKEFLLYLAGFVDGDGSIYAQITPTQGLKFKHRLSLWFNVTQKTQRRWFLDKLVDEIGVGYVYDSGSVSRYVLSQIKPLHNFLTQLQPFLKLKQKQANLVLKIIEQLPSAKESPDKFLEVCTWVDQIAALNDSKTRKTTSETVRAVLD

SEQ ID NO: 200 - protein, 344 aa, Artificial Sequence
  Synthesized
MNTKYNKEFLLYLAGFVDGDGSIFAYIQPAQNSKFKHLLKLVFTVTQKTQRRWFLDKLADEIGVGYVRDHGSVSYYTLSQIKPLHNFLTQLQPFLKLKQKQANLVLKIIEQLPSAKESPDKFLEVCTWVDQIAALNDSKTRKTTSETVRAVLDSLPGSVGGLSPSQASSAASSASSSPGSGISEALRAGAGSGTGYNKEFLLYLAGFVDGDGSIYAQITPTQGLKFKHRLSLWFNVTQKTQRRWFLDKLVDEIGVGYVYDSGSVSRYVLSKIKPLHNFLTQLQPFLKLKQKQANLVLKIIEQLPSAKESPDKFLEVCTWVDQIAALNDSKTRKTTSETVRAVLD

SEQ ID NO: 201 - protein, 344 aa, Artificial Sequence
  Synthesized
MNTKYNKEFLLYLAGFVDGDGSIYACIRPVQRSKFKHGLQLFFAVVQKTQRRWFLDKLVDEIGVGYVYDSGSVSRYILSEIKPLHNFLTQLQPFLKLKQKQANLVLKIIEQLPSAKESPDKFLEVCTWVDQIAALNDSKTRKTTSETVRAVLDSLPGSVGGLSPSQASSAASSASSSPGSGISEALRAGAGSGTGYNKEFLLYLAGFVDGDGSIYAYITPMQRRKFKHQLALVFAVTQKTQRRWFLDKLADEIGVGYVRDAGSVSQYVLSQIKPLHNFLTQLQPFLKLKQKQANLVLKIIEQLPSAKESPDKFLEVCTWVDQIAALNDSKTRKTTSETVRAVLD

SEQ ID NO: 202 - protein, 147 aa, Artificial Sequence
  Synthesized
KEFLLYLAGFVDGDGSIFAYIQPAQNSKFKHLLKLVFTVTQKTQRRWFLDKLVDEIGVGYVRDHGSVSYYTLSQIKPLHNFLTQLQPFLKLKQKQANLVLKIIEQLPSAKESPDKFLEVCTWVDQIAALNDSKTRKTTSETVRAVLD

SEQ ID NO: 203 - protein, 147 aa, Artificial Sequence
  Synthesized
KEFLLYLAGFVDGDGSIFAYIQPAQNSKFKHLLKLVFTVTQKTQRRWFLDKLADEIGVGYVRDAGSVSYYTLSQIKPLHNFLTQLQPFLKLKQKQANLVLKIIEQLPSAKESPDKFLEVCTWVDQIAALNDSKTRKTTSETVRAVLD

SEQ ID NO: 204 - protein, 147 aa, Artificial Sequence
  Synthesized
KEFLLYLAGFVDGDGSIFAYIQPAQNSKFKHLLKLVFTVTQKTQRRWFLDKLADEIGVGYVRDHGSVSYYTLSQIKPLHNFLTQLQPFLKLKQKQANLVLKIIEQLPSAKESPDKFLEVCTWVDQIAALNDSKTRKTTSETVRAVLD

SEQ ID NO: 205 - protein, 147 aa, Artificial Sequence
  Synthesized
KEFLLYLAGFVDGDGSIYAYITPMQRRKFKHQLALVFAVTQKTQRRWFLDKLADEIGVGYVRDAGSVSQYVLSQIKPLHNFLTQLQPFLKLKQKQANLVLKIIEQLPSAKESPDKFLEVCTWVDQIAALNDSKTRKTTSETVRAVLD

SEQ ID NO: 206 - protein, 147 aa, Artificial Sequence
  Synthesized
KEFLLYLAGFVDGDGSIYAQITPTQGLKFKHRLSLWFNVTQKTQRRWFLDKLVDEIGVGYVYDSGSVSRYILSQIKPLHNFLTQLQPFLKLKQKQANLVLKIIEQLPSAKESPDKFLEVCTWVDQIAALNDSKTRKTTSETVRAVLD

SEQ ID NO: 207 - protein, 147 aa, Artificial Sequence
  Synthesized
KEFLLYLAGFVDGDGSIYAQITPTQGLKFKHRLSLWFNVTQKTQRRWFLDKLVDEIGVGYVYDSGSVSRYVLSQIKPLHNFLTQLQPFLKLKQKQANLVLKIIEQLPSAKESPDKFLEVCTWVDQIAALNDSKTRKTTSETVRAVLD

SEQ ID NO: 208 - protein, 147 aa, Artificial Sequence
  Synthesized
KEFLLYLAGFVDGDGSIYAQITPTQGLKFKHRLSLWFNVTQKTQRRWFLDKLVDEIGVGYVYDSGSVSRYVLSKIKPLHNFLTQLQPFLKLKQKQANLVLKIIEQLPSAKESPDKFLEVCTWVDQIAALNDSKTRKTTSETVRAVLD

SEQ ID NO: 209 - protein, 147 aa, Artificial Sequence
  Synthesized
KEFLLYLAGFVDGDGSIYACIRPVQRSKFKHGLQLFFAVVQKTQRRWFLDKLVDEIGVGYVYDSGSVSRYILSEIKPLHNFLTQLQPFLKLKQKQANLVLKIIEQLPSAKESPDKFLEVCTWVDQIAALNDSKTRKTTSETVRAVLD

SEQ ID NO: 210 - protein, 354 aa, Artificial Sequence
  Synthesized
MNTKYNKEFLLYLAGFVDGDGSIYAQIKPRQQTKFKHDLRLSFAVDQKTQRRWFLDKLVDEIGVGYVYDYGSVSTYRLSQIKPLHNFLTQLQPFLKLKQKQANLVLKIIEQLPSAKESPDKFLEVCTWVDQIAALNDSKTRKTTSETVRAVLDSLPGSVGGLSPSQASSAASSASSSPGSGISEALRAGAGSGTGYNKEFLLYLAGFVDGDGSIYAMIRPRQDAKFKHTLRLWFAVAQKTQRRWFLDKLVDEIGVGYVTDWGSVSLYRLSQIKPLHNFLTQLQPFLKLKQKQANLVLKIIEQLPSAKESPDKFLEVCTWVDQIAALNDSKTRKTTSETVRAVLDSLSEKKKSSP

SEQ ID NO: 211 - protein, 354 aa, Artificial Sequence
  Synthesized
MNTKYNKEFLLYLAGFVDGDGSIWASINPVQPAKFKHRLRLFFGVFQKTQRRWFLDKLVDEIGVGYVYDDGSVSRYLLSKIKPLHNFLTQLQPFLKLKQKQANLVLKIIEQLPSAKESPDKFLEVCTWVDQIAALNDSKTRKTTSETVRAVLDSLPGSVGGLSPSQASSAASSASSSPGSGISEALRAGAGSGTGYNKEFLLYLAGFVDGDGSIYAEIKPRQDMKFKHALRLRFVVTQKTQRRWFLDKLVDEIGVGYVTDWGSVSQYRLSEIKPLHNFLTQLQPFLKLKQKQANLVLKIIEQLPSAKESPDKFLEVCTWVDQIAALNDSKTRKTTSETVRAVLDSLSEKKKSSP

SEQ ID NO: 212 - protein, 354 aa, Artificial Sequence
  Synthesized
MNTKYNKEFLLYLAGFVDGDGSIYATIAPLQGSKFKHRLRLHFSVDQKTQRRWFLDKLVDEIGVGYVYDYGSVSTYRLSEIKPLHNFLTQLQPFLKLKQKQANLVLKIIEQLPSAKESPDKFLEVCTWVDQIAALNDSKTRKTTSETVRAVLDSLPGSVGGLSPSQASSAASSASSSPGSGISEALRAGAGSGTGYNKEFLLYLAGFVDGDGSIYAMIRPRQDAKFKHTLRLWFAVAQKTQRRWFLDKLVDEIGVGYVTDWGSVSLYRLSQIKPLHNFLTQLQPFLKLKQKQANLVLKIIEQLPSAKESPDKFLEVCTWVDQIAALNDSKTRKTTSETVRAVLDSLSEKKKSSP

SEQ ID NO: 213 - protein, 354 aa, Artificial Sequence
  Synthesized
MNTKYNKEFLLYLAGFVDGDGSIYACITPRQCFKFKHQLRLAFIVTQKTQRRWFLDKLVDEIGVGYVTDHGSVSYYRLSEIKPLHNFLTQLQPFLKLKQKQANLVLKIIEQLPSAKESPDKFLEVCTWVDQIAALNDSKTRKTTSETVRAVLDSLPGSVGGLSPSQASSAASSASSSPGSGISEALRAGAGSGTGYNKEFLLYLAGFVDGDGSIWASINPVQPAKFKHRLRLFFGVFQKTQRRWFLDKLVDEIGVGYVYDDGSVSRYLLSEIKPLHNFLTQLQPFLKLKQKQANLVLKIIEQLPSAKESPDKFLEVCTWVDQIAALNDSKTRKTTSETVRAVLDSLSEKKKSSP

SEQ ID NO: 214 - protein, 147 aa, Artificial Sequence
  Synthesized
KEFLLYLAGFVDGDGSIYAQIKPRQQTKFKHDLRLSFAVDQKTQRRWFLDKLVDEIGVGYVYDYGSVSTYRLSQIKPLHNFLTQLQPFLKLKQKQANLVLKIIEQLPSAKESPDKFLEVCTWVDQIAALNDSKTRKTTSETVRAVLD

SEQ ID NO: 215 - protein, 147 aa, Artificial Sequence
  Synthesized
KEFLLYLAGFVDGDGSIWASINPVQPAKFKHRLRLFFGVFQKTQRRWFLDKLVDEIGVGYVYDDGSVSRYLLSKIKPLHNFLTQLQPFLKLKQKQANLVLKIIEQLPSAKESPDKFLEVCTWVDQIAALNDSKTRKTTSETVRAVLD

SEQ ID NO: 216 - protein, 147 aa, Artificial Sequence
  Synthesized
KEFLLYLAGFVDGDGSIYATIAPLQGSKFKHRLRLHFSVDQKTQRRWFLDKLVDEIGVGYVYDYGSVSTYRLSEIKPLHNFLTQLQPFLKLKQKQANLVLKIIEQLPSAKESPDKFLEVCTWVDQIAALNDSKTRKTTSETVRAVLD

SEQ ID NO: 217 - protein, 147 aa, Artificial Sequence
  Synthesized
KEFLLYLAGFVDGDGSIWASINPVQPAKFKHRLRLFFGVFQKTQRRWFLDKLVDEIGVGYVYDDGSVSRYLLSEIKPLHNFLTQLQPFLKLKQKQANLVLKIIEQLPSAKESPDKFLEVCTWVDQIAALNDSKTRKTTSETVRAVLD

SEQ ID NO: 218 - protein, 147 aa, Artificial Sequence
  Synthesized
KEFLLYLAGFVDGDGSIYAMIRPRQDAKFKHTLRLWFAVAQKTQRRWFLDKLVDEIGVGYVTDWGSVSLYRLSQIKPLHNFLTQLQPFLKLKQKQANLVLKIIEQLPSAKESPDKFLEVCTWVDQIAALNDSKTRKTTSETVRAVLD

SEQ ID NO: 219 - protein, 147 aa, Artificial Sequence
  Synthesized
KEFLLYLAGFVDGDGSIYAEIKPRQDMKFKHALRLRFVVTQKTQRRWFLDKLVDEIGVGYVTDWGSVSQYRLSEIKPLHNFLTQLQPFLKLKQKQANLVLKIIEQLPSAKESPDKFLEVCTWVDQIAALNDSKTRKTTSETVRAVLD

SEQ ID NO: 220 - protein, 147 aa, Artificial Sequence; identical to SEQ ID NO: 218
  Synthesized

SEQ ID NO: 221 - protein, 147 aa, Artificial Sequence
  Synthesized
KEFLLYLAGFVDGDGSIYACITPRQCFKFKHQLRLAFIVTQKTQRRWFLDKLVDEIGVGYVTDHGSVSYYRLSEIKPLHNFLTQLQPFLKLKQKQANLVLKIIEQLPSAKESPDKFLEVCTWVDQIAALNDSKTRKTTSETVRAVLD

SEQ ID NO: 222 - protein, 354 aa, Artificial Sequence
  Synthesized
MNTKYNKEFLLYLAGFVDGDGSIYARIWPAQQMKFKHQLYLTFRVYQKTQRRWFLDKLVDEIGVGYVADDGSVSYYQLSQIKPLHNFLTQLQPFLKLKQKQANLVLKIIEQLPSAKESPDKFLEVCTWVDQIAALNDSKTRKTTSETVRAVLDSLPGSVGGLSPSQASSAASSASSSPGSGISEALRAGAGSGTGYNKEFLLYLAGFVDGDGSIYARIQPRQDFKFKHQLLLTFNVSQKTQRRWFLDKLVDEIGAGYVCDGGGVSNYYLSQIKPLHNFLTQLQPFLKLKQKQANLVLKIIEQLPSAKESPDKFLEVCTWVDQIAALNDSKTRKTTSETVRAVLDSLSEKKKSSP

SEQ ID NO: 223 - protein, 354 aa, Artificial Sequence
  Synthesized
MNTKYNKEFLLYLAGFVDGDGSIYARIWPAQQMKFKHQLYLTFRVYQKTQRRWFLDKLVDEIGVGYVADDGSVSYYQLSQIKPLHNFLTQLQPFLKLKQKQANLVLKIIEQLPSAKESPDKFLEVCTWVDQIAALNDSKTRKTTSETVRAVLDSLPGSVGGLSPSQASSAASSASSSPGSGISEALRAGAGSGTGYNKEFLLYLAGFVDGDGSIYARIVPRQDFKFKHQLLLTFNVTQKTQRRWFLDKLVDEIGAGYVCDYGGVSNYYLSEIKPLHNFLTQLQPFLKLKQKQANLVLKIIEQLPSAKESPDKFLEVCTWVDQIAALNDSKTRKTTSETVRAVLDSLSEKKKSSP

SEQ ID NO: 224 - protein, 354 aa, Artificial Sequence
  Synthesized
MNTKYNKEFLLYLAGFVDGDGSIYARIWPAQQMKFKHQLYLTFRVYQKTQRRWFLDKLVDEIGVGYVADDGSVSYYQLSQIKPLHNFLTQLQPFLKLKQKQANLVLKIIEQLPSAKESPDKFLEVCTWVDQIAALNDSKTRKTTSETVRAVLDSLPGSVGGLSPSQASSAASSASSSPGSGISEALRAGAGSGTGYNKEFLLYLAGFVDGDGSIYARITPRQDFKFKHQLLLTFNVCQKTQRRWFLDKLVDEIGAGYVCDAGGVSNYYLSEIKPLHNFLTQLQPFLKLKQKQANLVLKIIEQLPSAKESPDKFLEVCTWVDQIAALNDSKTRKTTSETVRAVLDSLSEKKKSSP

SEQ ID NO: 225 - protein, 354 aa, Artificial Sequence
  Synthesized
MNTKYNKEFLLYLAGFVDGDGSIYARIWPAQQMKFKHQLYLTFRVYQKTQRRWFLDKLVDEIGVGYVADDGSVSYYQLSQIKPLHNFLTQLQPFLKLKQKQANLVLKIIEQLPSAKESPDKFLEVCTWVDQIAALNDSKTRKTTSETVRAVLDSLPGSVGGLSPSQASSAASSASSSPGSGISEALRAGAGSGTGYNKEFLLYLAGFVDGDGSIYARIVPRQDFKFKHQLLLTFNVTQKTQRRWFLDKLVDEIGAGYVCDHGGVSNYYLSEIKPLHNFLTQLQPFLKLKQKQANLVLKIIEQLPSAKESPDKFLEVCTWVDQIAALNDSKTRKTTSETVRAVLDSLSEKKKSSP

SEQ ID NO: 226 - protein, 147 aa, Artificial Sequence
  Synthesized
KEFLLYLAGFVDGDGSIYARIQPRQDFKFKHQLLLTFNVSQKTQRRWFLDKLVDEIGAGYVCDGGGVSNYYLSQIKPLHNFLTQLQPFLKLKQKQANLVLKIIEQLPSAKESPDKFLEVCTWVDQIAALNDSKTRKTTSETVRAVLD

SEQ ID NO: 227 - protein, 147 aa, Artificial Sequence
  Synthesized
KEFLLYLAGFVDGDGSIYARIVPRQDFKFKHQLLLTFNVTQKTQRRWFLDKLVDEIGAGYVCDYGGVSNYYLSEIKPLHNFLTQLQPFLKLKQKQANLVLKIIEQLPSAKESPDKFLEVCTWVDQIAALNDSKTRKTTSETVRAVLD

SEQ ID NO: 228 - protein, 147 aa, Artificial Sequence
  Synthesized
KEFLLYLAGFVDGDGSIYARITPRQDFKFKHQLLLTFNVCQKTQRRWFLDKLVDEIGAGYVCDAGGVSNYYLSEIKPLHNFLTQLQPFLKLKQKQANLVLKIIEQLPSAKESPDKFLEVCTWVDQIAALNDSKTRKTTSETVRAVLD

SEQ ID NO: 229 - protein, 147 aa, Artificial Sequence
  Synthesized
KEFLLYLAGFVDGDGSIYARIVPRQDFKFKHQLLLTFNVTQKTQRRWFLDKLVDEIGAGYVCDHGGVSNYYLSEIKPLHNFLTQLQPFLKLKQKQANLVLKIIEQLPSAKESPDKFLEVCTWVDQIAALNDSKTRKTTSETVRAVLD

SEQ ID NO: 230 - protein, 147 aa, Artificial Sequence
  Synthesized
KEFLLYLAGFVDGDGSIYARIWPAQQMKFKHQLYLTFRVYQKTQRRWFLDKLVDEIGVGYVADDGSVSYYQLSQIKPLHNFLTQLQPFLKLKQKQANLVLKIIEQLPSAKESPDKFLEVCTWVDQIAALNDSKTRKTTSETVRAVLD

SEQ ID NO: 231 - protein, 147 aa, Artificial Sequence; identical to SEQ ID NO: 230
  Synthesized

SEQ ID NO: 232 - protein, 147 aa, Artificial Sequence; identical to SEQ ID NO: 230
  Synthesized

SEQ ID NO: 233 - protein, 147 aa, Artificial Sequence; identical to SEQ ID NO: 230
  Synthesized

SEQ ID NO: 234 - protein, 354 aa, Artificial Sequence
  Synthesized
MNTKYNKEFLLYLAGFVDGDGSIYATIQPIQKVKFKHQLGLHFAVSQKTQRRWFLDKLVDEIGVGYVKDAGSVSYYMLSQIKPLHNFLTQLQPFLKLKQKQANLVLKIIEQLPSAKESPDKFLEVCTWVDQIAALNDSKTRKTTSETVRAVLDSLPGSVGGLSPSQASSAASSASSSPGSGISEALRAGAGSGTGYNKEFLLYLAGFVDGDGSIYASICPTQGHKFKHQLMLRFDVTQKTQRRWFLDKLVDEIGVGYVTDQGSVSRYRLSEIKPLHNFLTQLQPFLKLKQKQANLVLKIIEQLPSAKESPDKFLEVCTWVDQIAALNDSKTRKTTSETVRAVLDSLSEKKKSSP

SEQ ID NO: 235 - protein, 354 aa, Artificial Sequence
  Synthesized
MNTKYNKEFLLYLAGFVDGDGSIYATIQPIQKVKFKHQLGLHFAVSQKTQRRWFLDKLVDEIGVGYVKDAGSVSYYMLSEIKPLHNFLTQLQPFLKLKQKQANLVLKIIEQLPSAKESPDKFLEVCTWVDQIAALNDSKTRKTTSETVRAVLDSLPGSVGGLSPSQASSAASSASSSPGSGISEALRAGAGSGTGYNKEFLLYLAGFVDGDGSIYASIIPNQYGKFKHGLALRFDVTQKTQRRWFLDKLVDEIGVGYVTDQGSVSRYKLSQIKPLHNFLTQLQPFLKLKQKQANLVLKIIEQLPSAKESPDKFLEVCTWVDQIAALNDSKTRKTTSETVRAVLDSLSEKKKSSP

SEQ ID NO: 236 - protein, 354 aa, Artificial Sequence
  Synthesized
MNTKYNKEFLLYLAGFVDGDGSIYATIQPIQKVKFKHQLGLHFAVSQKTQRRWFLDKLVDEIGVGYVKDAGSVSYYMLSEIKPLHNFLTQLQPFLKLKQKQANLVLKIIEQLPSAKESPDKFLEVCTWVDQIAALNDSKTRKTTSETVRAVLDSLPGSVGGLSPSQASSAASSASSSPGSGISEALRAGAGSGTGYNKEFLLYLAGFVDGDGSIYASIVPHQSFKFKHQLALRFVVVQKTRRRWFLDKLVDEIGVGYVSDRGSVSDYRLSQIKPLHNFLTQLQPFLKLKQKQANLVLKIIEQLPSAKESPDKFLEVCTWVDQIAALNDSKTRKTTSETVRAVLDSLSEKKKSSP

SEQ ID NO: 237 - protein, 354 aa, Artificial Sequence
  Synthesized
MNTKYNKEFLLYLAGFVDGDGSIYASIIPNQYGKFKHGLALRFDVTQKTQRRWFLDKLVDEIGVGYVTDQGSVSRYKLSQIKPLHNFLTQLQPFLKLKQKQANLVLKIIEQLPSAKESPDKFLEVCTWVDQIAALNDSKTRKTTSETVRAVLDSLPGSVGGLSPSQASSAASSASSSPGSGISEALRAGAGSGTGYNKEFLLYLAGFVDGDGSIYATIQPIQKVKFKHQLGLHFAVSQKTQRRWFLDKLVDEIGVGYVKDAGSVSYYMLSQIKPLHNFLTQLQPFLKLKQKQANLVLKIIEQLPSAKESPDKFLEVCTWVDQIAALNDSKTRKTTSETVRAVLDSLSEKKKSSP

SEQ ID NO: 238 - protein, 147 aa, Artificial Sequence
  Synthesized
KEFLLYLAGFVDGDGSIYATIQPIQKVKFKHQLGLHFAVSQKTQRRWFLDKLVDEIGVGYVKDAGSVSYYMLSQIKPLHNFLTQLQPFLKLKQKQANLVLKIIEQLPSAKESPDKFLEVCTWVDQIAALNDSKTRKTTSETVRAVLD

SEQ ID NO: 239 - protein, 147 aa, Artificial Sequence
  Synthesized
KEFLLYLAGFVDGDGSIYATIQPIQKVKFKHQLGLHFAVSQKTQRRWFLDKLVDEIGVGYVKDAGSVSYYMLSEIKPLHNFLTQLQPFLKLKQKQANLVLKIIEQLPSAKESPDKFLEVCTWVDQIAALNDSKTRKTTSETVRAVLD

SEQ ID NO: 240 - protein, 147 aa, Artificial Sequence; identical to SEQ ID NO: 239
  Synthesized

SEQ ID NO: 241 - protein, 147 aa, Artificial Sequence; identical to SEQ ID NO: 238
  Synthesized

SEQ ID NO: 242 - protein, 147 aa, Artificial Sequence
  Synthesized
KEFLLYLAGFVDGDGSIYASICPTQGHKFKHQLMLRFDVTQKTQRRWFLDKLVDEIGVGYVTDQGSVSRYRLSEIKPLHNFLTQLQPFLKLKQKQANLVLKIIEQLPSAKESPDKFLEVCTWVDQIAALNDSKTRKTTSETVRAVLD

SEQ ID NO: 243 - protein, 147 aa, Artificial Sequence
  Synthesized
KEFLLYLAGFVDGDGSIYASIIPNQYGKFKHGLALRFDVTQKTQRRWFLDKLVDEIGVGYVTDQGSVSRYKLSQIKPLHNFLTQLQPFLKLKQKQANLVLKIIEQLPSAKESPDKFLEVCTWVDQIAALNDSKTRKTTSETVRAVLD

SEQ ID NO: 244 - protein, 147 aa, Artificial Sequence
  Synthesized
KEFLLYLAGFVDGDGSIYASIVPHQSFKFKHQLALRFVVVQKTRRRWFLDKLVDEIGVGYVSDRGSVSDYRLSQIKPLHNFLTQLQPFLKLKQKQANLVLKIIEQLPSAKESPDKFLEVCTWVDQIAALNDSKTRKTTSETVRAVLD

SEQ ID NO: 245 - protein, 147 aa, Artificial Sequence; identical to SEQ ID NO: 243
  Synthesized

SEQ ID NO: 246 - DNA, 2100 bp, Homo sapiens
actttcagagctgcagaatagctagagcagcaggggccctggcttttggaaactgacccgacctttattccagattctgccccactccgcagagctgtgtgaccttgggggattcccctaacctctctgagacgtggctttgttttctgtagggagaagataaaggtgacgcccattttgcggacctggtgtgaggattaaatgggaataacatagataaagtcttcagaacttcaaattagttcccctttcttcctttggggggtacaaagaaatatctgacccagttacgccacggcttgaaaggaggaaacccaaagaatggctgtggggatgaggaagattcctcaaggggaggacatggtatttaatgagggtcttgaagatgccaaggaagtggtagagggtgtttcacgaggagggaaccgtctgggcaaaggccaggaaggcggaaggggatcccttcagagtggctggtacgccgcatgtattaggggagatgaaagaggcaggccacgtccaagccatatttgtgttgctctccggagtttgtactttaggcttgaacttcccacacgtgttatttggcccacattgtgtttgaagaaactttgggattggttgccagtgcttaaaagttaggacttagaaaatggatttcctggcaggacgcggtggctcatgcccataatctcagcactttgggaggcctaggaaggtggatcacctgaggtccggagttcaagactaacctggccaacatggtgaaacccagtatctactaaaaaatacaaaaaaaaaaaaaaaagaagaagaagaagaagaaaataaagaaaagttagccgggcgtggtgtcgcgcgcctgtaatcccagctactccagaggctgcggcaggagaatcgcttgagcccgggaggcagaggttgcattaagccaagatcgcccaatgcactccggcctgggcgacagagcaagactccgtctcaaaaaataataataataaataaaaataaaaaataaaatggatttcccagcatctctggaaaaataggcaagtgtggccatgatggtccttagatctcctctaggaaagcagacatttattacttggcttctgtgcactatctgagctgccacgtattgggcttccacccctgcctgtgtggacagcatgggttgtcagcagagttgtgttttgttttgtttttttgagacagagtttccctcttgttgcccaggctggagtgcagtggctcagtctcagctcactgcaacctctgcctcctgggttcaagtgattctcctgcctcagcctcccgagtagctgggattatcggctaattttgtatttttagtagagacagatttctccatgttggtcaggctggtctcgaactcccaacctcaggtgatccgcccacctcgccctcccaaagtgctggaattacaggcgtgagccaccgcgtctggccatcagcagagtttttaatttaggagaatgacaagaggtggtacagttttttagatggtacctggtggctgttaagggctattgactgacaaacacacccaacttggcgctgccgcccaggaggtggacactgggtttctggatagatggttagcaacctctgtcaccagctgggcctctttttttctatactgaattaatcacatttgtttaacctgtctgttccatagttcccttgcacatcttgggtatttgaggagttgggtgggtggcagtggcaactggggccaccatcctgtttaattattttaaagccctgactgtcctggattgaccctaagctccccctggtctccaaaattcatcagaaactgagttcacttgaaggcctcttccccacccttttctccaccccttgcatctacttctaaagcagctgttcaacagaaacagaatgggagccacacacataattctacattttctagttaaaaagaaaaaaaaatcattttcaacaatatatttattcaacctagtacatacaaaatattatcattccaacatgtaatcagtattttaaaaatcagtaatgagaccaggcacggtggctcacgactgtaatcccagg

SEQ ID NO: 247 - DNA, 906 bp, Artificial Sequence
  Synthesized
ccagttacgccacggcttgaaaggaggaaacccaaagaatggctgtggggatgaggaagattcctcaaggggaggacatggtatttaatgagggtcttgaagatgccaaggaagtggtagagggtgtttcacgaggagggaaccgtctgggcaaaggccaggaaggcggaaggggatcccttcagagtggctggtacgccgcatgtattaggggagatgaaagaggcaggccacgtccaagccatatttgtgttgctctccggagtttgtactttaggcttgaacttcccacacgtgttatttggcccacattgtgtttgaagaaactttgggattggttgccagtgcttaaaagttaggacttagaaaatggatttcctggcaggacgcggtggctcatgcccataatctcagcactttgggaggcctaggaaggtggatcacctgaggtccggagttcaagactaacctggccaacatggtgaaacccagtatctactaaaaaatacaaaaaaaaaaaaaaaagaagaagaagaagaagaaaataaagaaaagttagccgggcgtggtgtcgcgcgcctgtaatcccagctactccagaggctgcggcaggagaatcgcttgagcccgggaggcagaggttgcattaagccaagatcgcccaatgcactccggcctgggcgacagagcaagactccgtctcaaaaaataataataataaataaaaataaaaaataaaatggatttcccagcatctctggaaaaataggcaagtgtggccatgatggtccttagatctcctctaggaaagcagacatttattacttggcttctgtgcactatctgagctgccacgtattgggcttccacccctgcctgtgtggacagcatgggttgtcagcagag

SEQ ID NO: 248 - DNA, 907 bp, Artificial Sequence
  Synthesized
ccagttacgccacggcttgaaaggaggaaacccaaagaatggctgtggggatgaggaagattcctcaaggggaggacatggtatttaatgagggtcttgaagatgccaaggaagtggtagagggtgtttcacgaggagggaaccgtctgggcaaaggccaggaaggcggaaggggatcccttcagagtggctggtacgccgcatgtattaggggagatgaaagaggcaggccacgtccaagccatatttgtgttgctctccggagtttgtactttaggcttaaacattcccacacgtgttatttggcccacattgtgtttgaagaaactttgggattggttgccagtgcttaaaagttaggacttagaaaatggatttcctggcaggacgcggtggctcatgcccataatctcagcactttgggaggcctaggaaggtggatcacctgaggtccggagttcaagactaacctggccaacatggtgaaacccagtatctactaaaaaatacaaaaaaaaaaaaaaaagaagaagaagaagaagaaaataaagaaaagttagccgggcgtggtgtcgcgcgcctgtaatcccagctactccagaggctgcggcaggagaatcgcttgagcccgggaggcagaggttgcattaagccaagatcgcccaatgcactccggcctgggcgacagagcaagactccgtctcaaaaaataataataataaataaaaataaaaaataaaatggatttcccagcatctctggaaaaataggcaagtgtggccatgatggtccttagatctcctctaggaaagcagacatttattacttggcttctgtgcactatctgagctgccacgtattgggcttccacccctgcctgtgtggacagcatgggttgtcagcagag

SEQ ID NO: 249 - DNA, 928 bp, Artificial Sequence
  Synthesized
ccagttacgccacggcttgaaaggaggaaacccaaagaatggctgtggggatgaggaagattcctcaaggggaggacatggtatttaatgagggtcttgaagatgccaaggaaggggtggaaacacaggcatgtccacaaccagggtgtttcacgaggagggaaccgtctgggcaaaggccaggaaggcggaaggggatcccttcagagtggctggtacgccgcatgtattaggggagatgaaagaggcaggccacgtccaagccatatttgtgttgctctccggagtttgtactttaggcttgaacttcccacacgtgttatttggcccacattgtgtttgaagaaactttgggattggttgccagtgcttaaaagttaggacttagaaaatggatttcctggcaggacgcggtggctcatgcccataatctcagcactttgggaggcctaggaaggtggatcacctgaggtccggagttcaagactaacctggccaacatggtgaaacccagtatctactaaaaaatacaaaaaaaaaaaaaaaagaagaagaagaagaagaaaataaagaaaagttagccgggcgtggtgtcgcgcgcctgtaatcccagctactccagaggctgcggcaggagaatcgcttgagcccgggaggcagaggttgcattaagccaagatcgcccaatgcactccggcctgggcgacagagcaagactccgtctcaaaaaataataataataaataaaaataaaaaataaaatggatttcccagcatctctggaaaaataggcaagtgtggccatgatggtccttagatctcctctaggaaagcagacatttattacttggcttctgtgcactatctgagctgccacgtattgggcttccacccctgcctgtgtggacagcatgggttgtcagcagag

SEQ ID NO: 250 - DNA, 906 bp, Artificial Sequence; identical to SEQ ID NO: 247
  Synthesized